European Patent Application EP 4 335 873 A1, published March 13, 2024. Title: ANTI-CLAUDIN 18.2 ANTIBODY AND ANTIBODY-DRUG CONJUGATE THEREOF. Applicant: REMEGEN CO., LTD. The sequence listing filed with the application follows.

SEQUENCE LISTING (34 sequences)

SEQ ID NO: 1 - protein, 119 aa, Artificial sequence
  Heavy chain variable region
QVQLVQSGAEVKKPGASVKVSCKASGYAFTNYLIEWVRQAPGQGLEWMGLINPGSGGTNYNEKFKGRVTMTRDTSTSTVYMELSSLRSEDTAVYYCARGGYYGNSFAYWGQGTLVTVSS

SEQ ID NO: 2 - protein, 113 aa, Artificial sequence
  Light chain variable region
DIVMTQSPLSLPVTPGEPASISCKSSQSLLNSGNQKNYLTWYLQKPGQSPQLLIYWASTRESGVPDRFSGSGSGTDFTLKISRVEAEDVGVYYCQNAYYYPYTFGGGTKVEIK

SEQ ID NO: 3 - protein, 7 aa, Artificial sequence
  CDR of heavy chain
GYAFTNY

SEQ ID NO: 4 - protein, 10 aa, Artificial sequence
  CDR of heavy chain
GYAFTNYLIE

SEQ ID NO: 5 - protein, 5 aa, Artificial sequence
  CDR of heavy chain
NYLIE

SEQ ID NO: 6 - protein, 6 aa, Artificial sequence
  CDR of heavy chain
TNYLIE

SEQ ID NO: 7 - protein, 8 aa, Artificial sequence
  CDR of heavy chain
GYAFTNYL

SEQ ID NO: 8 - protein, 6 aa, Artificial sequence
  CDR of heavy chain
NPGSGG

SEQ ID NO: 9 - protein, 10 aa, Artificial sequence
  CDR of heavy chain
LINPGSGGTN

SEQ ID NO: 10 - protein, 17 aa, Artificial sequence
  CDR of heavy chain
LINPGSGGTNYNEKFKG

SEQ ID NO: 11 - protein, 13 aa, Artificial sequence
  CDR of heavy chain
WMGLINPGSGGTN

SEQ ID NO: 12 - protein, 8 aa, Artificial sequence
  CDR of heavy chain
INPGSGGT

SEQ ID NO: 13 - protein, 10 aa, Artificial sequence
  CDR of heavy chain
GGYYGNSFAY

SEQ ID NO: 14 - protein, 10 aa, Artificial sequence
  CDR of heavy chain
GGYYGNSFAY

SEQ ID NO: 15 - protein, 10 aa, Artificial sequence
  CDR of heavy chain
GGYYGNSFAY

SEQ ID NO: 16 - protein, 11 aa, Artificial sequence
  CDR of heavy chain
ARGGYYGNSFA

SEQ ID NO: 17 - protein, 12 aa, Artificial sequence
  CDR of heavy chain
ARGGYYGNSFAY

SEQ ID NO: 18 - protein, 17 aa, Artificial sequence
  CDR of light chain
KSSQSLLNSGNQKNYLT

SEQ ID NO: 19 - protein, 17 aa, Artificial sequence
  CDR of light chain
KSSQSLLNSGNQKNYLT

SEQ ID NO: 20 - protein, 17 aa, Artificial sequence
  CDR of light chain
KSSQSLLNSGNQKNYLT

SEQ ID NO: 21 - protein, 13 aa, Artificial sequence
  CDR of light chain
LNSGNQKNYLTWY

SEQ ID NO: 22 - protein, 12 aa, Artificial sequence
  CDR of light chain
QSLLNSGNQKNY

SEQ ID NO: 23 - protein, 7 aa, Artificial sequence
  CDR of light chain
WASTRES

SEQ ID NO: 24 - protein, 7 aa, Artificial sequence
  CDR of light chain
WASTRES

SEQ ID NO: 25 - protein, 7 aa, Artificial sequence
  CDR of light chain
WASTRES

SEQ ID NO: 26 - protein, 10 aa, Artificial sequence
  CDR of light chain
LLIYWASTRE

SEQ ID NO: 27 - protein, 3 aa, Artificial sequence
  CDR of light chain
WAS

SEQ ID NO: 28 - protein, 9 aa, Artificial sequence
  CDR of light chain
QNAYYYPYT

SEQ ID NO: 29 - protein, 9 aa, Artificial sequence
  CDR of light chain
QNAYYYPYT

SEQ ID NO: 30 - protein, 9 aa, Artificial sequence
  CDR of light chain
QNAYYYPYT

SEQ ID NO: 31 - protein, 8 aa, Artificial sequence
  CDR of light chain
QNAYYYPY

SEQ ID NO: 32 - protein, 9 aa, Artificial sequence
  CDR of light chain
QNAYYYPYT

SEQ ID NO: 33 - protein, 449 aa, Artificial sequence
  Heavy chain
QVQLVQSGAEVKKPGASVKVSCKASGYAFTNYLIEWVRQAPGQGLEWMGLINPGSGGTNYNEKFKGRVTMTRDTSTSTVYMELSSLRSEDTAVYYCARGGYYGNSFAYWGQGTLVTVSSASTKGPSVFPLAPSSKSTSGGTAALGCLVKDYFPEPVTVSWNSGALTSGVHTFPAVLQSSGLYSLSSVVTVPSSSLGTQTYICNVNHKPSNTKVDKKVEPKSCDKTHTCPPCPAPELLGGPSVFLFPPKPKDTLMISRTPEVTCVVVDVSHEDPEVKFNWYVDGVEVHNAKTKPREEQYNSTYRVVSVLTVLHQDWLNGKEYKCKVSNKALPAPIEKTISKAKGQPREPQVYTLPPSREEMTKNQVSLTCLVKGFYPSDIAVEWESNGQPENNYKTTPPVLDSDGSFFLYSKLTVDKSRWQQGNVFSCSVMHEALHNHYTQKSLSLSPGK

SEQ ID NO: 34 - protein, 220 aa, Artificial sequence
  Light chain
DIVMTQSPLSLPVTPGEPASISCKSSQSLLNSGNQKNYLTWYLQKPGQSPQLLIYWASTRESGVPDRFSGSGSGTDFTLKISRVEAEDVGVYYCQNAYYYPYTFGGGTKVEIKRTVAAPSVFIFPPSDEQLKSGTASVVCLLNNFYPREAKVQWKVDNALQSGNSQESVTEQDSKDSTYSLSSTLTLSKADYEKHKVYACEVTHQGLSSPVTKSFNRGEC